European Patent Application EP 4 516 300 A2, published March 5, 2025. Title: Rational Therapeutic Targeting of Oncogenic Immune Signaling States in Myeloid Malignancies via the Ubiquitin Conjugating Enzyme UBE2N. Applicant: CHILDREN'S HOSPITAL MEDICAL CENTER. Application EP, filed June 15, 2020. The sequence listing filed with the application follows.

SEQUENCE LISTING (34 sequences)

SEQ ID NO: 1 - RNA, 22 nt, synthetic construct
  modified_base 1: mod_base = OTHER; note = thymine
  modified_base 4: mod_base = OTHER; note = thymine
  modified_base 6: mod_base = OTHER; note = thymine
  modified_base 17: mod_base = OTHER; note = thymine
  misc_feature 1..22: note = UBE2N forward primer sequence
  source 1..22: mol_type = other RNA
tgatgtagcggagcagtggaag

SEQ ID NO: 2 - RNA, 22 nt, synthetic construct
  modified_base 9: mod_base = OTHER; note = thymine
  modified_base 11..12: mod_base = OTHER; note = thymine
  misc_feature 1..22: note = UBE2N reverse primer sequence
  source 1..22: mol_type = other RNA
ggaggaagtcttggcagaacag

SEQ ID NO: 3 - RNA, 21 nt, synthetic construct
  modified_base 8: mod_base = OTHER; note = thymine
  modified_base 13: mod_base = OTHER; note = thymine
  modified_base 15: mod_base = OTHER; note = thymine
  modified_base 17..18: mod_base = OTHER; note = thymine
  modified_base 21: mod_base = OTHER; note = thymine
  misc_feature 1..21: note = FOS forward primer sequence
  source 1..21: mol_type = other RNA
ccggggatagcctctcttact

SEQ ID NO: 4 - RNA, 19 nt, synthetic construct
  modified_base 6: mod_base = OTHER; note = thymine
  modified_base 10: mod_base = OTHER; note = thymine
  modified_base 18: mod_base = OTHER; note = thymine
  misc_feature 1..19: note = FOS reverse primer sequence
  source 1..19: mol_type = other RNA
ccaggtccgtgcagaagtc

SEQ ID NO: 5 - RNA, 21 nt, synthetic construct
  modified_base 1: mod_base = OTHER; note = thymine
  modified_base 7: mod_base = OTHER; note = thymine
  misc_feature 1..21: note = JUN forward primer sequence
  source 1..21: mol_type = other RNA
tccaagtgccgaaaaaggaag

SEQ ID NO: 6 - RNA, 21 nt, synthetic construct
  modified_base 5..6: mod_base = OTHER; note = thymine
  modified_base 8: mod_base = OTHER; note = thymine
  modified_base 13..15: mod_base = OTHER; note = thymine
  modified_base 21: mod_base = OTHER; note = thymine
  misc_feature 1..21: note = JUN reverse primer sequence
  source 1..21: mol_type = other RNA
cgagttctgagctttcaaggt

SEQ ID NO: 7 - RNA, 21 nt, synthetic construct
  modified_base 7: mod_base = OTHER; note = thymine
  modified_base 10: mod_base = OTHER; note = thymine
  misc_feature 1..21: note = JUNB forward primer sequence
  source 1..21: mol_type = other RNA
acaaactcctgaaaccgagcc

SEQ ID NO: 8 - RNA, 21 nt, synthetic construct
  modified_base 8: mod_base = OTHER; note = thymine
  modified_base 20: mod_base = OTHER; note = thymine
  misc_feature 1..21: note = JUNB reverse primer sequence
  source 1..21: mol_type = other RNA
cgagccctgaccagaaaagta

SEQ ID NO: 9 - RNA, 21 nt, synthetic construct
  modified_base 3: mod_base = OTHER; note = thymine
  modified_base 7: mod_base = OTHER; note = thymine
  modified_base 10: mod_base = OTHER; note = thymine
  modified_base 19: mod_base = OTHER; note = thymine
  modified_base 21: mod_base = OTHER; note = thymine
  misc_feature 1..21: note = IL6 forward primer sequence
  source 1..21: mol_type = other RNA
ggtacatcctcgacggcatct

SEQ ID NO: 10 - RNA, 21 nt, synthetic construct
  modified_base 2: mod_base = OTHER; note = thymine
  modified_base 6: mod_base = OTHER; note = thymine
  modified_base 8..10: mod_base = OTHER; note = thymine
  modified_base 13: mod_base = OTHER; note = thymine
  modified_base 16..18: mod_base = OTHER; note = thymine
  misc_feature 1..21: note = IL6 reverse primer sequence
  source 1..21: mol_type = other RNA
gtgcctctttgctgctttcac

SEQ ID NO: 11 - RNA, 23 nt, synthetic construct
  modified_base 3: mod_base = OTHER; note = thymine
  modified_base 5: mod_base = OTHER; note = thymine
  modified_base 7: mod_base = OTHER; note = thymine
  modified_base 11: mod_base = OTHER; note = thymine
  modified_base 13: mod_base = OTHER; note = thymine
  modified_base 16: mod_base = OTHER; note = thymine
  modified_base 20: mod_base = OTHER; note = thymine
  modified_base 22..23: mod_base = OTHER; note = thymine
  misc_feature 1..23: note = IL1B forward primer sequence
  source 1..23: mol_type = other RNA
aatctgtacctgtcctgcgtgtt

SEQ ID NO: 12 - RNA, 26 nt, synthetic construct
  modified_base 1: mod_base = OTHER; note = thymine
  modified_base 5: mod_base = OTHER; note = thymine
  modified_base 8..12: mod_base = OTHER; note = thymine
  modified_base 17: mod_base = OTHER; note = thymine
  modified_base 19: mod_base = OTHER; note = thymine
  modified_base 24: mod_base = OTHER; note = thymine
  modified_base 26: mod_base = OTHER; note = thymine
  misc_feature 1..26: note = IL1B reverse primer sequence
  source 1..26: mol_type = other RNA
tgggtaatttttgggatctacactct

SEQ ID NO: 13 - RNA, 20 nt, synthetic construct
  modified_base 1: mod_base = OTHER; note = thymine
  modified_base 3..4: mod_base = OTHER; note = thymine
  modified_base 6: mod_base = OTHER; note = thymine
  modified_base 18: mod_base = OTHER; note = thymine
  misc_feature 1..20: note = TNF forward primer sequence
  source 1..20: mol_type = other RNA
tcttctcgaaccccgagtga

SEQ ID NO: 14 - RNA, 19 nt, synthetic construct
  modified_base 3: mod_base = OTHER; note = thymine
  modified_base 5: mod_base = OTHER; note = thymine
  modified_base 8: mod_base = OTHER; note = thymine
  misc_feature 1..19: note = TNF reverse primer sequence
  source 1..19: mol_type = other RNA
cctctgatggcaccaccag

SEQ ID NO: 15 - RNA, 20 nt, synthetic construct
  modified_base 2: mod_base = OTHER; note = thymine
  modified_base 4..5: mod_base = OTHER; note = thymine
  modified_base 12..13: mod_base = OTHER; note = thymine
  modified_base 16..17: mod_base = OTHER; note = thymine
  modified_base 20: mod_base = OTHER; note = thymine
  misc_feature 1..20: note = Actin forward primer sequence
  source 1..20: mol_type = other RNA
ctcttccagccttccttcct

SEQ ID NO: 16 - RNA, 20 nt, synthetic construct
  modified_base 6: mod_base = OTHER; note = thymine
  modified_base 8: mod_base = OTHER; note = thymine
  modified_base 10..11: mod_base = OTHER; note = thymine
  modified_base 16: mod_base = OTHER; note = thymine
  misc_feature 1..20: note = Actin reverse primer sequence
  source 1..20: mol_type = other RNA
agcactgtgttggcgtacag

SEQ ID NO: 17 - RNA, 58 nt, synthetic construct
  modified_base 6: mod_base = OTHER; note = thymine
  modified_base 11: mod_base = OTHER; note = thymine
  modified_base 13: mod_base = OTHER; note = thymine
  modified_base 15: mod_base = OTHER; note = thymine
  modified_base 20: mod_base = OTHER; note = thymine
  modified_base 24: mod_base = OTHER; note = thymine
  modified_base 27: mod_base = OTHER; note = thymine
  modified_base 32: mod_base = OTHER; note = thymine
  modified_base 34..35: mod_base = OTHER; note = thymine
  modified_base 38: mod_base = OTHER; note = thymine
  modified_base 43: mod_base = OTHER; note = thymine
  modified_base 45: mod_base = OTHER; note = thymine
  modified_base 50: mod_base = OTHER; note = thymine
  modified_base 53..57: mod_base = OTHER; note = thymine
  misc_feature 1..58: note = UBE2N template oligonucleotide shUBE2N-2
  source 1..58: mol_type = other RNA
ccggctaggctatatgccatgaatactcgagtattcatggcatatagcctagtttttg

SEQ ID NO: 18 - RNA, 58 nt, synthetic construct
  modified_base 12..13: mod_base = OTHER; note = thymine
  modified_base 22: mod_base = OTHER; note = thymine
  modified_base 24: mod_base = OTHER; note = thymine
  modified_base 27: mod_base = OTHER; note = thymine
  modified_base 34: mod_base = OTHER; note = thymine
  modified_base 36..37: mod_base = OTHER; note = thymine
  modified_base 39..40: mod_base = OTHER; note = thymine
  modified_base 47..48: mod_base = OTHER; note = thymine
  modified_base 50: mod_base = OTHER; note = thymine
  modified_base 52..57: mod_base = OTHER; note = thymine
  misc_feature 1..58: note = UBE2N template oligonucleotide shUBE2N-3
  source 1..58: mol_type = other RNA
ccggagacaagttgggaagaatatgctcgagcatattcttcccaacttgtcttttttg

SEQ ID NO: 19 - RNA, 57 nt, synthetic construct
  modified_base 7: mod_base = OTHER; note = thymine
  modified_base 14..16: mod_base = OTHER; note = thymine
  modified_base 18: mod_base = OTHER; note = thymine
  modified_base 22: mod_base = OTHER; note = thymine
  modified_base 24..25: mod_base = OTHER; note = thymine
  modified_base 27: mod_base = OTHER; note = thymine
  modified_base 37: mod_base = OTHER; note = thymine
  modified_base 44: mod_base = OTHER; note = thymine
  modified_base 48: mod_base = OTHER; note = thymine
  modified_base 53..57: mod_base = OTHER; note = thymine
  misc_feature 1..57: note = UBE2N template oligonucleotide shUBE2N-1
  source 1..57: mol_type = other RNA
ccgggctgaggcatttgtgagtcttctcgagaagactcacaaatgcctcagcttttt

SEQ ID NO: 20 - RNA, 57 nt, synthetic construct
  modified_base 13: mod_base = OTHER; note = thymine
  modified_base 27: mod_base = OTHER; note = thymine
  modified_base 32..33: mod_base = OTHER; note = thymine
  modified_base 36: mod_base = OTHER; note = thymine
  modified_base 39: mod_base = OTHER; note = thymine
  modified_base 41..42: mod_base = OTHER; note = thymine
  modified_base 45: mod_base = OTHER; note = thymine
  modified_base 47..48: mod_base = OTHER; note = thymine
  modified_base 50..51: mod_base = OTHER; note = thymine
  modified_base 53..57: mod_base = OTHER; note = thymine
  misc_feature 1..57: note = Non-silencing control shControl
  source 1..57: mol_type = other RNA
ccggcaacaagatgaagagcaccaactcgagttggtgctcttcatcttgttgttttt

SEQ ID NO: 21 - protein, 11 aa, synthetic construct
  REGION 1..11: note = UBE2N Ub conjugation peptide with ubiquinated diglycine (UGG) motif
IYHPNVDKLGR

SEQ ID NO: 22 - protein, 12 aa, synthetic construct
  REGION 1..12: note = UBE2N Ub conjugation peptide with ubiquinated diglycine (UGG) motif
FMTKIYHPNVDK

SEQ ID NO: 23 - protein, 10 aa, synthetic construct
  REGION 1..10: note = UBE2N Ub conjugation peptide with ubiquinated diglycine (UGG) motif
DKWSPALQIR

SEQ ID NO: 24 - protein, 12 aa, synthetic construct
  REGION 1..12: note = UBE2N Ub conjugation peptide with ubiquinated diglycine (UGG) motif
IYHPNVDKLGRI

SEQ ID NO: 25 - protein, 12 aa, synthetic construct
  REGION 1..12: note = UBE2N Ub conjugation peptide with ubiquinated diglycine (UGG) motif
FMTKIYHPNVDK

SEQ ID NO: 26 - protein, 12 aa, synthetic construct
  REGION 1..12: note = UBE2N Ub conjugation peptide with ubiquinated diglycine (UGG) motif
VSFELFADKVPK

SEQ ID NO: 27 - protein, 13 aa, synthetic construct
  REGION 1..13: note = UBE2N Ub conserved site peptide with ubiquinated diglycine (UGG) motif
CCLTYCFNKPEDK

SEQ ID NO: 28 - protein, 16 aa, synthetic construct
  REGION 1..16: note = UBE2N Ub conserved site peptide with ubiquinated diglycine (UGG) motif
TLEVEPSDTIENVKAK

SEQ ID NO: 29 - protein, 13 aa, synthetic construct
  REGION 1..13: note = UBE2N Ub conserved site peptide with ubiquinated diglycine (UGG) motif
LKYYKVDENGKSR

SEQ ID NO: 30 - protein, 13 aa, synthetic construct
  REGION 1..13: note = UBE2N Ub-protein transferase activity peptide with ubiquinated diglycine (UGG) motif
LVCPDEGFYKSGK

SEQ ID NO: 31 - protein, 9 aa, synthetic construct
  REGION 1..9: note = UBE2N Ub-like protein ligase binding site with ubiquinated diglycine (UGG) motif
HTPLSKLMK

SEQ ID NO: 32 - protein, 18 aa, synthetic construct
  REGION 1..18: note = UBE2N Ub-like protein ligase binding site with ubiquinated diglycine (UGG) motif
LIYSGKQMNDEKTAADYK

SEQ ID NO: 33 - protein, 18 aa, synthetic construct
  REGION 1..18: note = UBE2N Ub-like protein ligase binding site with ubiquinated diglycine (UGG) motif
LIYSGKQMNDEKTAADYK

SEQ ID NO: 34 - protein, 11 aa, synthetic construct
  REGION 1..11: note = UBE2N Ub interacting motif with ubiquinated diglycine (UGG) motif
CNYKEHWFTVR